European Patent Specification EP 3 577 136 B1, published August 5, 2026. Title: INHIBITION OF PLATELET AGGREGATION USING ANTI-HUMAN GPVI ANTIBODIES. Applicant: ACTICOR BIOTECH UNIVERSITÉ PARIS DIDEROT - PARIS 7 UNIVERSITÉ PARIS XIII INSTITUT NATIONAL DE LA SANTÉ ET DE LA RECHERCHE MÉDICALE (INSERM) UNIVERSITÉ PARIS-SUD 11 Billiald Philippe Martine JANDROT-PERRUS Gilles AVENARD. The sequence listing filed with the application follows.

SEQUENCE LISTING (27 sequences)

SEQ ID NO: 1 - protein, 10 aa, Artificial Sequence
  VH-CDR1
GYTFTSYNMH

SEQ ID NO: 2 - protein, 17 aa, Artificial Sequence
  VH-CDR2
GIYPGNGDTSYNQKFQG

SEQ ID NO: 3 - protein, 11 aa, Artificial Sequence
  VH-CDR3
GTVVGDWYFDV

SEQ ID NO: 4 - protein, 16 aa, Artificial Sequence
  VL-CDR1
RSSQSLENSNGNTYLN

SEQ ID NO: 5 - protein, 7 aa, Artificial Sequence
  VL-CDR2
RVSNRFS

SEQ ID NO: 6 - protein, 9 aa, Artificial Sequence
  VL-CDR3
LQLTHVPWT

SEQ ID NO: 7 - protein, 120 aa, Artificial Sequence
  Heavy chain variable region
QVQLVQSGAEVKKPGASVKVSCKASGYTFTSYNMHWVRQAPGQGLEWMGGIYPGNGDTSYNQKFQGRVTMTRDTSTSTVYMELSSLRSEDTAVYYCARGTVVGDWYFDVWGQGTLVTVSS

SEQ ID NO: 8 - protein, 113 aa, Artificial Sequence
  Light chain variable region
DIQMTQSPSSLSASVGDRVTITCRSSQSLENSNGNTYLNWYQQKPGKAPKLLIYRVSNRFSGVPSRFSGSGSGTDFTFTISSLQPEDIATYYCLQLTHVPWTFGQGTKVEITR

SEQ ID NO: 9 - protein, 113 aa, Artificial Sequence
  Light chain variable region
DIQMTQSPSSLSASVGDRVTITCSASQSLENSNGNTYLNWYQQKPGKAPKLLIYRVSNRFSGVPSRFSGSGSGTDFTLTISSLQPEDFATYYCLQLTHVPWTFGQGTKVEIKR

SEQ ID NO: 10 - DNA, 360 bp, Artificial Sequence
  Heavy chain variable region
caggttcagctggttcagtcaggggctgaggtgaagaagcctggagcctcagtgaaggtgtcctgcaaggcttctggctacacatttaccagttacaatatgcactgggtaagacaggctcctggacagggcctggaatggatgggaggtatttatccaggaaatggtgatacttcctacaatcagaagttccagggccgagttactatgactcgggacacttccacctctacagtgtacatggagctcagcagcctgagatctgaggacaccgcggtctattactgtgcaagaggcaccgtggtcggcgactggtacttcgatgtgtggggccaaggcaccctggtcaccgtgagcagt

SEQ ID NO: 11 - DNA, 339 bp, Artificial Sequence
  Light chain variable region
gacatccagatgacccagagcccaagcagcctgagcgccagcgtgggtgacagagtgaccatcacctgtagaagtagtcagagccttgagaacagcaacggaaacacctacctgaattggtaccagcagaagccaggtaaggctccaaagctgctgatctacagagtttccaaccgattctctggtgtgccaagcagattcagcggtagcggtagcggtaccgacttcaccttcaccatcagcagcctccagccagaggacatcgccacctactactgcctccagctgactcatgtcccatggaccttcggtcagggcaccaaggtggagatcacccgg

SEQ ID NO: 12 - DNA, 339 bp, Artificial Sequence
  Light chain variable region
gacatccagatgacccagagcccaagcagcctgagcgccagcgtgggtgacagagtgaccatcacctgtagtgccagtcagagccttgagaacagcaacggaaacacctacctgaattggtaccagcagaagccaggtaaggctccaaagctgctgatctacagagtttccaaccgattctctggtgtgccaagcagattcagcggtagcggtagcggtaccgacttcaccctcaccatcagcagcctccagccagaggacttcgccacctactactgcctccagctgactcatgtcccatggaccttcggtcagggcaccaaggtggagatcaaacgc

SEQ ID NO: 13 - protein, 339 aa, Homo sapiens
MSPSPTALFCLGLCLGRVPAQSGPLPKPSLQALPSSLVPLEKPVTLRCQGPPGVDLYRLEKLSSSRYQDQAVLFIPAMKRSLAGRYRCSYQNGSLWSLPSDQLELVATGVFAKPSLSAQPGPAVSSGGDVTLQCQTRYGFDQFALYKEGDPAPYKNPERWYRASFPIITVTAAHSGTYRCYSFSSRDPYLWSAPSDPLELVVTGTSVTPSRLPTEPPSSVAEFSEATAELTVSFTNKVFTTETSRSITTSPKESDSPAGPARQYYTKGNLVRICLGAVILIILAGFLAEDWHSRRKRLRHRGRAVQRPLPPLPPLPQTRKSHGGQDGGRQDVHSRGLCS

SEQ ID NO: 14 - DNA, 321 bp, Artificial Sequence
  Heavy chain constant region
gcctccaccaagggtccctcagtcttcccactggcaccctcctccaagagcacctctggtggcacagctgccctgggctgcctggtcaaggactacttcccagaaccagtgactgtgtcatggaactcaggcgccctgaccagcggcgtgcacaccttccctgctgtcttgcagtcctcaggactctactccctcagcagcgtggtgaccgtgccctccagcagcttgggcacccagacctacatctgcaacgtgaatcacaagcccagcaacaccaaggtggacaagaaagtcgagcctaagtcatgcgacaagactcac

SEQ ID NO: 15 - DNA, 318 bp, Artificial Sequence
  Light chain constant region
actgtggctgcaccaagtgtgttcatcttcccacctagcgatgagcagttgaaatctggaactgcctctgtcgtgtgcctcctgaacaacttctacccacgggaggccaaggtacagtggaaggtggataacgccctccaatccggtaactcccaggagagtgtcacagagcaagatagcaaggacagcacctacagcctcagcagcaccctgactctgagcaaagcagactacgagaagcacaaggtctacgcctgcgaagtcacccatcagggcctgagttcccctgtcacaaagagcttcaaccggggagagtgt

SEQ ID NO: 16 - DNA, 66 bp, Artificial Sequence
  Signal peptide
atggatatgcgtgtaccagctcaactacttggacttctattgctttggcttcgtggtgctagatgt

SEQ ID NO: 17 - DNA, 57 bp, Artificial Sequence
  Signal peptide
atggactggacttggagaatcctattcttggttgctgcagctacaggtgctcattca

SEQ ID NO: 18 - DNA, 762 bp, Artificial Sequence
  Heavy chain
gcggccgccaccatggactggacttggagaatcctattcttggttgctgcagctacaggtgctcattcacaggttcagctggttcagtcaggggctgaggtgaagaagcctggagcctcagtgaaggtgtcctgcaaggcttctggctacacatttaccagttacaatatgcactgggtaagacaggctcctggacagggcctggaatggatgggaggtatttatccaggaaatggtgatacttcctacaatcagaagttccagggccgagttactatgactcgggacacttccacctctacagtgtacatggagctcagcagcctgagatctgaggacaccgcggtctattactgtgcaagaggcaccgtggtcggcgactggtacttcgatgtgtggggccaaggcaccctggtcaccgtgagcagtgcctccaccaagggtccctcagtcttcccactggcaccctcctccaagagcacctctggtggcacagctgccctgggctgcctggtcaaggactacttcccagaaccagtgactgtgtcatggaactcaggcgccctgaccagcggcgtgcacaccttccctgctgtcttgcagtcctcaggactctactccctcagcagcgtggtgaccgtgccctccagcagcttgggcacccagacctacatctgcaacgtgaatcacaagcccagcaacaccaaggtggacaagaaagtcgagcctaagtcatgcgacaagactcactgatgaggatcc

SEQ ID NO: 19 - DNA, 742 bp, Artificial Sequence
  Light chain
gacgtcaccatggatatgcgtgtaccagctcaactacttggacttctattgctttggcttcgtggtgctagatgtgacatccagatgacccagagcccaagcagcctgagcgccagcgtgggtgacagagtgaccatcacctgtagaagtagtcagagccttgagaacagcaacggaaacacctacctgaattggtaccagcagaagccaggtaaggctccaaagctgctgatctacagagtttccaaccgattctctggtgtgccaagcagattcagcggtagcggtagcggtaccgacttcaccttcaccatcagcagcctccagccagaggacatcgccacctactactgcctccagctgactcatgtcccatggaccttcggtcagggcaccaaggtggagatcacccggactgtggctgcaccaagtgtgttcatcttcccacctagcgatgagcagttgaaatctggaactgcctctgtcgtgtgcctcctgaacaacttctacccacgggaggccaaggtacagtggaaggtggataacgccctccaatccggtaactcccaggagagtgtcacagagcaagatagcaaggacagcacctacagcctcagcagcaccctgactctgagcaaagcagactacgagaagcacaaggtctacgcctgcgaagtcacccatcagggcctgagttcccctgtcacaaagagcttcaaccggggagagtgttgatgatatc

SEQ ID NO: 20 - DNA, 742 bp, Artificial Sequence
  Light chain
gacgtcaccatggatatgcgtgtaccagctcaactacttggacttctattgctttggcttcgtggtgctagatgtgacatccagatgacccagagcccaagcagcctgagcgccagcgtgggtgacagagtgaccatcacctgtagtgccagtcagagccttgagaacagcaacggaaacacctacctgaattggtaccagcagaagccaggtaaggctccaaagctgctgatctacagagtttccaaccgattctctggtgtgccaagcagattcagcggtagcggtagcggtaccgacttcaccctcaccatcagcagcctccagccagaggacttcgccacctactactgcctccagctgactcatgtcccatggaccttcggtcagggcaccaaggtggagatcaaacgcactgtggctgcaccaagtgtgttcatcttcccacctagcgatgagcagttgaaatctggaactgcctctgtcgtgtgcctcctgaacaacttctacccacgggaggccaaggtacagtggaaggtggataacgccctccaatccggtaactcccaggagagtgtcacagagcaagatagcaaggacagcacctacagcctcagcagcaccctgactctgagcaaagcagactacgagaagcacaaggtctacgcctgcgaagtcacccatcagggcctgagttcccctgtcacaaagagcttcaaccggggagagtgttgatgatatc

SEQ ID NO: 21 - protein, 4 aa, Artificial Sequence
  CDR-L3 - Residues after
  SITE 3: X is any amino acid
FGXG

SEQ ID NO: 22 - protein, 4 aa, Artificial Sequence
  CDR-H1 - Residues before
  SITE 2: X is any amino acid
  SITE 3: X is any amino acid
  SITE 4: X is any amino acid
CXXX

SEQ ID NO: 23 - protein, 5 aa, Artificial Sequence
  CDR-H2 - Residues before
LEWIG

SEQ ID NO: 24 - protein, 4 aa, Artificial Sequence
  CDR-H3 - Residues after
  SITE 3: X is any amino acid
WGXG

SEQ ID NO: 25 - protein, 527 aa, Homo sapiens
SYQVICRDEKTQMIYQQHQSWLRPVLRSNRVEYCWCNSGRAQCHSVPVKSCSEPRCFNGGTCQQALYFSDFVCQCPEGFAGKCCEIDTRATCYEDQGISYRGTWSTAESGAECTNWNSSALAQKPYSGRRPDAIRLGLGNHNYCRNPDRDSKPWCYVFKAGKYSSEFCSTPACSEGNSDCYFGNGSAYRGTHSLTESGASCLPWNSMILIGKVYTAQNPSAQALGLGKHNYCRNPDGDAKPWCHVLKNRRLTWEYCDVPSCSTCGLRQYSQPQFRIKGGLFADIASHPWQAAIFAKHRRSPGERFLCGGILISSCWILSAAHCFQERFPPHHLTVILGRTYRVVPGEEEQKFEVEKYIVHKEFDDDTYDNDIALLQLKSDSSRCAQESSVVRTVCLPPADLQLPDWTECELSGYGKHEALSPFYSERLKEAHVRLYPSSRCTSQHLLNRTVTDNMLCAGDTRSGGPQANLHDACQGDSGGPLVCLNDGRMTLVGIISWGLGCGQKDVPGVYTKVTNYLDWIRDNMRP

SEQ ID NO: 26 - protein, 275 aa, Homo sapiens
SYQVICRDEKTQMIYQQHQSWLRPVLRSNRVEYCWCNSGRAQCHSVPVKSCSEPRCFNGGTCQQALYFSDFVCQCPEGFAGKCCEIDTRATCYEDQGISYRGTWSTAESGAECTNWNSSALAQKPYSGRRPDAIRLGLGNHNYCRNPDRDSKPWCYVFKAGKYSSEFCSTPACSEGNSDCYFGNGSAYRGTHSLTESGASCLPWNSMILIGKVYTAQNPSAQALGLGKHNYCRNPDGDAKPWCHVLKNRRLTWEYCDVPSCSTCGLRQYSQPQFR

SEQ ID NO: 27 - protein, 252 aa, Homo sapiens
IKGGLFADIASHPWQAAIFAKHRRSPGERFLCGGILISSCWILSAAHCFQERFPPHHLTVILGRTYRVVPGEEEQKFEVEKYIVHKEFDDDTYDNDIALLQLKSDSSRCAQESSVVRTVCLPPADLQLPDWTECELSGYGKHEALSPFYSERLKEAHVRLYPSSRCTSQHLLNRTVTDNMLCAGDTRSGGPQANLHDACQGDSGGPLVCLNDGRMTLVGIISWGLGCGQKDVPGVYTKVTNYLDWIRDNMRP